European Patent Application EP 4 530 297 A1, published April 2, 2025. Title: ANTI-ASGR1 MONOCLONAL ANTIBODY AND USE THEREOF. Applicant: WUHAN UNIVERSITY. The sequence listing filed with the application follows.

SEQUENCE LISTING (38 sequences)

SEQ ID NO: 1 - protein, 291 aa, Homo sapiens
MTKEYQDLQHLDNEESDHHQLRKGPPPPQPLLQRLCSGPRLLLLSLGLSLLLLVVVCVIGSQNSQLQEELRGLRETFSNFTASTEAQVKGLSTQGGNVGRKMKSLESQLEKQQKDLSEDHSSLLLHVKQFVSDLRSLSCQMAALQGNGSERTCCPVNWVEHERSCYWFSRSGKAWADADNYCRLEDAHLVVVTSWEEQKFVQHHIGPVNTWMGLHDQNGPWKWVDGTDYETGFKNWRPEQPDDWYGHGLGGGEDCAHFTDDGRWNDDVCQRPYRWVCETELDKASQEPPLL

SEQ ID NO: 2 - protein, 150 aa, Homo sapiens
AALQGNGSERTCCPVNWVEHERSCYWFSRSGKAWADADNYCRLEDAHLVVVTSWEEQKFVQHHIGPVNTWMGLHDQNGPWKWVDGTDYETGFKNWRPEQPDDWYGHGLGGGEDCAHFTDDGRWNDDVCQRPYRWVCETELDKASQEPPLL

SEQ ID NO: 3 - protein, 93 aa, Homo sapiens
RLEDAHLVVVTSWEEQKFVQHHIGPVNTWMGLHDQNGPWKWVDGTDYETGFKNWRPEQPDDWYGHGLGGGEDCAHFTDDGRWNDDVCQRPYRW

SEQ ID NO: 4 - protein, 8 aa, Rabbit
QSVYNNKN

SEQ ID NO: 5 - skipped

SEQ ID NO: 6 - protein, 13 aa, Rabbit
QGEFSCSSADCCA

SEQ ID NO: 7 - protein, 9 aa, Rabbit
GFSFSGSLW

SEQ ID NO: 8 - protein, 9 aa, Rabbit
IYVGSSGST

SEQ ID NO: 9 - protein, 20 aa, Rabbit
ARRYTDAYGGYPAGSFVFKL

SEQ ID NO: 10 - protein, 6 aa, Rabbit
QKISNE

SEQ ID NO: 11 - skipped

SEQ ID NO: 12 - protein, 15 aa, Rabbit
QCTYGSSNIVNYGGA

SEQ ID NO: 13 - protein, 8 aa, Rabbit
GFSLSSNA

SEQ ID NO: 14 - protein, 7 aa, Rabbit
IVSSGAA

SEQ ID NO: 15 - protein, 5 aa, Rabbit
VRGNL

SEQ ID NO: 16 - protein, 6 aa, Rabbit
ESISSY

SEQ ID NO: 17 - skipped

SEQ ID NO: 18 - protein, 13 aa, Rabbit
QSNYGTTSSTYDT

SEQ ID NO: 19 - protein, 9 aa, Rabbit
GFSFNKKYY

SEQ ID NO: 20 - protein, 9 aa, Rabbit
IYAGSSGST

SEQ ID NO: 21 - protein, 19 aa, Rabbit
ARGYYYYNGYVYYGYGMDL

SEQ ID NO: 22 - protein, 6 aa, Rabbit
ESISSY

SEQ ID NO: 23 - skipped

SEQ ID NO: 24 - protein, 12 aa, Rabbit
QQGYSGNNLDNA

SEQ ID NO: 25 - protein, 8 aa, Rabbit
GFSLSSYA

SEQ ID NO: 26 - protein, 7 aa, Rabbit
IYASGST

SEQ ID NO: 27 - protein, 12 aa, Rabbit
ARGDDSYTTDDL

SEQ ID NO: 28 - protein, 112 aa, Rabbit
QVLTQTPSPVSAAVGGTVTINCQASQSVYNNKNLGWYQQKPGQPPKLLIYYASDLASGVPSRFKGSGSGKQFTLTISDVQCDDAATYYCQGEFSCSSADCCAFGGGTEVVVK

SEQ ID NO: 29 - protein, 127 aa, Rabbit
QSLEESGGDLVKPGATMTLTCKASGFSFSGSLWICWVRQAPGKGLEWIACIYVGSSGSTYYASWAKGRFTISTTSSTTVTLQMTSLTAADTATYFCARRYTDAYGGYPAGSFVFKLWGPGTLVTVSS

SEQ ID NO: 30 - protein, 113 aa, Rabbit
DVVMTQTPASVEAAVGGTVTIKCQASQKISNELSWYQQKPGQPPKRLIYRASTLESGVPSRFKGSGSGTEFTLTISDLECADAATYYCQCTYGSSNIVNYGGAFGGGTEVVVK

SEQ ID NO: 31 - protein, 108 aa, Rabbit
QSVEESGGRLVTPGTPLTLTCTVSGFSLSSNAINWVRQAPGKGLEWIGYIVSSGAAYYASWAKGRFTISKTSTTVDLSITSPTTEDTATYFCVRGNLWGPGTLVTVSS

SEQ ID NO: 32 - protein, 111 aa, Rabbit
DIVMTQTPASVEAAVGGTITINCQASESISSYLSWYQQKPGQRPKLLIYQASKLESGVPSRFKGSGSGTEYTLTISDLECADAATYYCQSNYGTTSSTYDTFGGGTEVVVK

SEQ ID NO: 33 - protein, 127 aa, Rabbit
QEQLEESGGDLVKPEGSLTLTCTASGFSFNKKYYMCWVRQAPGKGLEWIACIYAGSSGSTYYASWVNGRFTISQTSSTTVTLQMTSLTAADTATYFCARGYYYYNGYVYYGYGMDLWGPGTLVTVSS

SEQ ID NO: 34 - protein, 110 aa, Rabbit
AYDMTQTPASVEVAVGGTVTIKCQASESISSYLNWYQQKPGQRPKVLIYDASDLASGVSSRFKGSGSGTQFTLTISGVQCDDAATYYCQQGYSGNNLDNAFGGGTEVVVK

SEQ ID NO: 35 - protein, 115 aa, Rabbit
QSVEESGGRLVTPGTPLTLTCTVSGFSLSSYAMSWVRQAPGKGLEYIGIIYASGSTYYASWAKGRFTISKTSTTVDLKMTSPTTEDTATYFCARGDDSYTTDDLWGPGTLVTVSS

SEQ ID NO: 36 - DNA, 1310 bp, Homo sapiens
  source 1..1310: mol_type = other DNA
acacagacacgcagacacagagacaccggggcccagggccctcctatggaccctgcccgctcccctcccattgtccacggctgtccgcccacccccattctccaagcttcagccccctccttagttcggcatctgcacagcactgaagaacctgggaatcagaccctgagaccctgagcaatcccaggtccagcgccagccctatcatgaccaaggagtatcaagaccttcagcatctggacaatgaggagagtgaccaccatcagctcagaaaagggccacctcctccccagcccctcctgcagcgtctctgctccggacctcgcctcctcctgctctccctgggcctcagcctcctgctgcttgtggttgtctgtgtgatcggatcccaaaactcccagctgcaggaggagctgcggggcctgagagagacgttcagcaacttcacagcgagcacggaggcccaggtcaagggcttgagcacccagggaggcaatgtgggaagaaagatgaagtcgctagagtcccagctggagaaacagcagaaggacctgagtgaagatcactccagcctgctgctccacgtgaagcagttcgtgtctgacctgcggagcctgagctgtcagatggcggcgctccagggcaatggctcagaaaggacctgctgcccggtcaactgggtggagcacgagcgcagctgctactggttctctcgctccgggaaggcctgggctgacgccgacaactactgccggctggaggacgcgcacctggtggtggtcacgtcctgggaggagcagaaatttgtccagcaccacataggccctgtgaacacctggatgggcctccacgaccaaaacgggccctggaagtgggtggacgggacggactacgagacgggcttcaagaactggaggccggagcagccggacgactggtacggccacgggctcggaggaggcgaggactgtgcccacttcaccgacgacggccgctggaacgacgacgtctgccagaggccctaccgctgggtctgcgagacagagctggacaaggccagccaggagccacctctcctttaatttatttcttcaatgcctcgacctgccgcaggggtccgggattgggaatccgcccatctgggggcctcttctgctttctcgggaattttcatctaggattttaagggaaggggaaggatagggtgatgttccgaaggtgaggagcttgaaacccgtggcgctttctgcagtttgcaggttatcattgtgaactttttttttttaagagtaaaaagaaatatacctaaa

SEQ ID NO: 37 - protein, 330 aa, Homo sapiens [sequence omitted]

SEQ ID NO: 38 - protein, 107 aa, Homo sapiens [sequence omitted]